European Patent Application EP 4 378 487 A2, published June 5, 2024. Title: MODIFIED FACTOR IX, AND COMPOSITIONS, METHODS AND USES FOR GENE TRANSFER TO CELLS, ORGANS AND TISSUES. Applicant: THE CHILDREN'S HOSPITAL OF PHILADELPHIA. Application EP. The sequence listing filed with the application follows.

SEQUENCE LISTING (27 sequences)

SEQ ID NO: 1 - protein, 738 aa, unidentified
  source 1..738: note = Adeno-associated Virus
MAADGYLPDWLEDNLSEGIREWWDLKPGAPKPKANQQKQDNGRGLVLPGYKYLGPFNGLDKGEPVNAADAAALEHDKAYDQQLQAGDNPYLRYNHADAEFQERLQEDTSFGGNLGRAVFQAKKRVLEPLGLVESPVKTAPGKKRPVEPSPQRSPDSSTGIGKKGQQPAKKRLNFGQTGDSESVPDPQPIGEPPAGPSGLGSGTMAAGGGAPMADNNEGADGVGSSSGNWHCDSTWLGDRVITTSTRTWALPTYNNHLYKQISNGTSGGSTNDNTYFGYSTPWGYFDFNRFHCHFSPRDWQRLINNNWGFRPKRLNFKLFNIQVKEVTQNEGTKTIANNLTSTIQVFTDSEYQLPYVLGSAHQGCLPPFPADVFMIPQYGYLTLNNGSQAVGRSSFYCLEYFPSQMLRTGNNFEFSYNFEDVPFHSSYAHSQSLDRLMNPLIDQYLYYLSRTQSTGGTAGTQQLLFSQAGPNNMSAQAKNWLPGPCYRQQRVSTTLSQNNNSNFAWTGATKYHLNGRDSLVNPGVAMATHKDDEERFFPSSGVLMFGKQGAGKDNVDYSSVMLTSEEEIKTTNPVATEQYGVVADNLQQQNAAPIVGAVNSQGALPGMVWQNRDVYLQGPIWAKIPHTDGNFHPSPLMGGFGLKHPPPQILIKNTPVPADPPTTFNQAKLASFITQYSTGQVSVEIEWELQKENSKRWNPEIQYTSNYYKSTNVDFAVNTEGTYSEPRPIGTRYLTRNL

SEQ ID NO: 2 - protein, 601 aa, unidentified
  source 1..601: note = Adeno-associated Virus
TAPGKKRPVEPSPQRSPDSSTGIGKKGQQPAKKRLNFGQTGDSESVPDPQPIGEPPAGPSGLGSGTMAAGGGAPMADNNEGADGVGSSSGNWHCDSTWLGDRVITTSTRTWALPTYNNHLYKQISNGTSGGSTNDNTYFGYSTPWGYFDFNRFHCHFSPRDWQRLINNNWGFRPKRLNFKLFNIQVKEVTQNEGTKTIANNLTSTIQVFTDSEYQLPYVLGSAHQGCLPPFPADVFMIPQYGYLTLNNGSQAVGRSSFYCLEYFPSQMLRTGNNFEFSYNFEDVPFHSSYAHSQSLDRLMNPLIDQYLYYLSRTQSTGGTAGTQQLLFSQAGPNNMSAQAKNWLPGPCYRQQRVSTTLSQNNNSNFAWTGATKYHLNGRDSLVNPGVAMATHKDDEERFFPSSGVLMFGKQGAGKDNVDYSSVMLTSEEEIKTTNPVATEQYGVVADNLQQQNAAPIVGAVNSQGALPGMVWQNRDVYLQGPIWAKIPHTDGNFHPSPLMGGFGLKHPPPQILIKNTPVPADPPTTFNQAKLASFITQYSTGQVSVEIEWELQKENSKRWNPEIQYTSNYYKSTNVDFAVNTEGTYSEPRPIGTRYLTRNL

SEQ ID NO: 3 - protein, 535 aa, unidentified
  source 1..535: note = Adeno-associated Virus
MAAGGGAPMADNNEGADGVGSSSGNWHCDSTWLGDRVITTSTRTWALPTYNNHLYKQISNGTSGGSTNDNTYFGYSTPWGYFDFNRFHCHFSPRDWQRLINNNWGFRPKRLNFKLFNIQVKEVTQNEGTKTIANNLTSTIQVFTDSEYQLPYVLGSAHQGCLPPFPADVFMIPQYGYLTLNNGSQAVGRSSFYCLEYFPSQMLRTGNNFEFSYNFEDVPFHSSYAHSQSLDRLMNPLIDQYLYYLSRTQSTGGTAGTQQLLFSQAGPNNMSAQAKNWLPGPCYRQQRVSTTLSQNNNSNFAWTGATKYHLNGRDSLVNPGVAMATHKDDEERFFPSSGVLMFGKQGAGKDNVDYSSVMLTSEEEIKTTNPVATEQYGVVADNLQQQNAAPIVGAVNSQGALPGMVWQNRDVYLQGPIWAKIPHTDGNFHPSPLMGGFGLKHPPPQILIKNTPVPADPPTTFNQAKLASFITQYSTGQVSVEIEWELQKENSKRWNPEIQYTSNYYKSTNVDFAVNTEGTYSEPRPIGTRYLTRNL

SEQ ID NO: 4 - protein, 738 aa, unidentified
  source 1..738: note = Adeno-associated Virus
MAADGYLPDWLEDNLSEGIREWWDLKPGAPKPKANQQKQDNGRGLVLPGYKYLGPFNGLDKGEPVNAADAAALEHDKAYDQQLQAGDNPYLRYNHADAEFQERLQEDTSFGGNLGRAVFQAKKRVLEPLGLVESPVKTAPGKKRPVEPSPQRSPDSSTGIGKKGQQPAKKRLNFGQTGDSESVPDPQPIGEPPAAPSGVGPNTMAAGGGAPMADNNEGADGVGSSSGNWHCDSTWLGDRVITTSTRTWALPTYNNHLYKQISNGTSGGSTNDNTYFGYSTPWGYFDFNRFHCHFSPRDWQRLINNNWGFRPKRLNFKLFNIQVKEVTQNEGTKTIANNLTSTIQVFTDSEYQLPYVLGSAHQGCLPPFPADVFMIPQYGYLTLNNGSQAVGRSSFYCLEYFPSQMLRTGNNFEFSYNFEDVPFHSSYAHSQSLDRLMNPLIDQYLYYLSRTQSTGGTAGTQQLLFSQAGPNNMSAQAKNWLPGPCYRQQRVSTTLSQNNNSNFAWTGATKYHLNGRDSLVNPGVAMATHKDDEERFFPSSGVLMFGKQGAGKDNVDYSSVMLTSEEEIKTTNPVATEQYGVVADNLQQQNAAPIVGAVNSQGALPGMVWQNRDVYLQGPIWAKIPHTDGNFHPSPLMGGFGLKHPPPQILIKNTPVPADPPTTFNQAKLASFITQYSTGQVSVEIEWELQKENSKRWNPEIQYTSNYYKSTNVDFAVNTEGTYSEPRPIGTRYLTRNL

SEQ ID NO: 5 - protein, 738 aa, unidentified
  source 1..738: note = Adeno-associated Virus
MAADGYLPDWLEDNLSEGIREWWDLKPGAPKPKANQQRQDNGRGLVLPGYRYLGPFNGLDKGEPVNAADAAALEHDRAYDQQLQAGDNPYLRYNHADAEFQERLQEDTSFGGNLGRAVFQAKKRVLEPLGLVESPVRTAPGKKRPVEPSPQRSPDSSTGIGKKGQQPARKRLNFGQTGDSESVPDPQPIGEPPAAPSGVGPNTMAAGGGAPMADNNEGADGVGSSSGNWHCDSTWLGDRVITTSTRTWALPTYNNHLYRQISNGTSGGSTNDNTYFGYSTPWGYFDFNRFHCHFSPRDWQRLINNNWGFRPKRLNFKLFNIQVKEVTQNEGTRTIANNLTSTIQVFTDSEYQLPYVLGSAHQGCLPPFPADVFMIPQYGYLTLNNGSQAVGRSSFYCLEYFPSQMLRTGNNFEFSYNFEDVPFHSSYAHSQSLDRLMNPLIDQYLYYLSRTQSTGGTAGTQQLLFSQAGPNNMSAQAKNWLPGPCYRQQRVSTTLSQNNNSNFAWTGATKYHLNGRDSLVNPGVAMATHRDDEERFFPSSGVLMFGRQGAGRDNVDYSSVMLTSEEEIRTTNPVATEQYGVVADNLQQQNAAPIVGAVNSQGALPGMVWQNRDVYLQGPIWAKIPHTDGNFHPSPLMGGFGLKHPPPQILIKNTPVPADPPTTFNQAKLASFITQYSTGQVSVEIEWELQKENSKRWNPEIQYTSNYYKSTNVDFAVNTEGTYSEPRPIGTRYLTRNL

SEQ ID NO: 6 - protein, 738 aa, unidentified
  source 1..738: note = Adeno-associated Virus
MAADGYLPDWLEDNLSEGIREWWDLKPGAPKPKANQQRQDNGRGLVLPGYRYLGPFNGLDKGEPVNAADAAALEHDRAYDQQLQAGDNPYLRYNHADAEFQERLQEDTSFGGNLGRAVFQAKKRVLEPLGLVESPVRTAPGKKRPVEPSPQRSPDSSTGIGKRGQQPARKRLNFGQTGDSESVPDPQPIGEPPAAPSGVGPNTMAAGGGAPMADNNEGADGVGSSSGNWHCDSTWLGDRVITTSTRTWALPTYNNHLYRQISNGTSGGSTNDNTYFGYSTPWGYFDFNRFHCHFSPRDWQRLINNNWGFRPKRLNFKLFNIQVKEVTQNEGTRTIANNLTSTIQVFTDSEYQLPYVLGSAHQGCLPPFPADVFMIPQYGYLTLNNGSQAVGRSSFYCLEYFPSQMLRTGNNFEFSYNFEDVPFHSSYAHSQSLDRLMNPLIDQYLYYLSRTQSTGGTAGTQQLLFSQAGPNNMSAQAKNWLPGPCYRQQRVSTTLSQNNNSNFAWTGATKYHLNGRDSLVNPGVAMATHRDDEERFFPSSGVLMFGKQGAGRDNVDYSSVMLTSEEEIRTTNPVATEQYGVVADNLQQQNAAPIVGAVNSQGALPGMVWQNRDVYLQGPIWAKIPHTDGNFHPSPLMGGFGLKHPPPQILIKNTPVPADPPTTFNQAKLASFITQYSTGQVSVEIEWELQKENSKRWNPEIQYTSNYYKSTNVDFAVNTEGTYSEPRPIGTRYLTRNL

SEQ ID NO: 7 - protein, 738 aa, unidentified
  source 1..738: note = Adeno-associated Virus
MAADGYLPDWLEDNLSEGIREWWDLKPGAPKPKANQQRQDNGRGLVLPGYRYLGPFNGLDKGEPVNAADAAALEHDRAYDQQLQAGDNPYLRYNHADAEFQERLQEDTSFGGNLGRAVFQAKKRVLEPLGLVESPVRTAPGKKRPVEPSPQRSPDSSTGIGKRGQQPAKKRLNFGQTGDSESVPDPQPIGEPPAAPSGVGPNTMAAGGGAPMADNNEGADGVGSSSGNWHCDSTWLGDRVITTSTRTWALPTYNNHLYRQISNGTSGGSTNDNTYFGYSTPWGYFDFNRFHCHFSPRDWQRLINNNWGFRPKRLNFKLFNIQVKEVTQNEGTRTIANNLTSTIQVFTDSEYQLPYVLGSAHQGCLPPFPADVFMIPQYGYLTLNNGSQAVGRSSFYCLEYFPSQMLRTGNNFEFSYNFEDVPFHSSYAHSQSLDRLMNPLIDQYLYYLSRTQSTGGTAGTQQLLFSQAGPNNMSAQAKNWLPGPCYRQQRVSTTLSQNNNSNFAWTGATKYHLNGRDSLVNPGVAMATHRDDEERFFPSSGVLMFGRQGAGRDNVDYSSVMLTSEEEIRTTNPVATEQYGVVADNLQQQNAAPIVGAVNSQGALPGMVWQNRDVYLQGPIWAKIPHTDGNFHPSPLMGGFGLKHPPPQILIKNTPVPADPPTTFNQAKLASFITQYSTGQVSVEIEWELQKENSKRWNPEIQYTSNYYKSTNVDFAVNTEGTYSEPRPIGTRYLTRNL

SEQ ID NO: 8 - protein, 738 aa, unidentified
  source 1..738: note = Adeno-associated Virus
MAADGYLPDWLEDNLSEGIREWWDLKPGAPKPKANQQRQDNGRGLVLPGYRYLGPFNGLDKGEPVNAADAAALEHDRAYDQQLQAGDNPYLRYNHADAEFQERLQEDTSFGGNLGRAVFQAKKRVLEPLGLVESPVRTAPGKKRPVEPSPQRSPDSSTGIGKRGQQPAKKRLNFGQTGDSESVPDPQPIGEPPAAPSGVGPNTMAAGGGAPMADNNEGADGVGSSSGNWHCDSTWLGDRVITTSTRTWALPTYNNHLYRQISNGTSGGSTNDNTYFGYSTPWGYFDFNRFHCHFSPRDWQRLINNNWGFRPKRLNFKLFNIQVKEVTQNEGTRTIANNLTSTIQVFTDSEYQLPYVLGSAHQGCLPPFPADVFMIPQYGYLTLNNGSQAVGRSSFYCLEYFPSQMLRTGNNFEFSYNFEDVPFHSSYAHSQSLDRLMNPLIDQYLYYLSRTQSTGGTAGTQQLLFSQAGPNNMSAQAKNWLPGPCYRQQRVSTTLSQNNNSNFAWTGATKYHLNGRDSLVNPGVAMATHRDDEERFFPSSGVLMFGKQGAGRDNVDYSSVMLTSEEEIRTTNPVATEQYGVVADNLQQQNAAPIVGAVNSQGALPGMVWQNRDVYLQGPIWAKIPHTDGNFHPSPLMGGFGLKHPPPQILIKNTPVPADPPTTFNQARLASFITQYSTGQVSVEIEWELQKENSKRWNPEIQYTSNYYKSTNVDFAVNTEGTYSEPRPIGTRYLTRNL

SEQ ID NO: 9 - protein, 738 aa, unidentified
  source 1..738: note = Adeno-associated Virus
MAADGYLPDWLEDNLSEGIREWWDLKPGAPKPKANQQRQDNGRGLVLPGYRYLGPFNGLDKGEPVNAADAAALEHDRAYDQQLQAGDNPYLRYNHADAEFQERLQEDTSFGGNLGRAVFQAKKRVLEPLGLVESPVRTAPGKKRPVEPSPQRSPDSSTGIGKKGQQPAKKRLNFGQTGDSESVPDPQPIGEPPAAPSGVGPNTMAAGGGAPMADNNEGADGVGSSSGNWHCDSTWLGDRVITTSTRTWALPTYNNHLYRQISNGTSGGSTNDNTYFGYSTPWGYFDFNRFHCHFSPRDWQRLINNNWGFRPKRLNFKLFNIQVKEVTQNEGTRTIANNLTSTIQVFTDSEYQLPYVLGSAHQGCLPPFPADVFMIPQYGYLTLNNGSQAVGRSSFYCLEYFPSQMLRTGNNFEFSYNFEDVPFHSSYAHSQSLDRLMNPLIDQYLYYLSRTQSTGGTAGTQQLLFSQAGPNNMSAQAKNWLPGPCYRQQRVSTTLSQNNNSNFAWTGATKYHLNGRDSLVNPGVAMATHRDDEERFFPSSGVLMFGRQGAGRDNVDYSSVMLTSEEEIRTTNPVATEQYGVVADNLQQQNAAPIVGAVNSQGALPGMVWQNRDVYLQGPIWAKIPHTDGNFHPSPLMGGFGLKHPPPQILIKNTPVPADPPTTFNQARLASFITQYSTGQVSVEIEWELQKENSKRWNPEIQYTSNYYKSTNVDFAVNTEGTYSEPRPIGTRYLTRNL

SEQ ID NO: 10 - DNA, 1386 bp, unidentified
  source 1..1386: mol_type = other DNA; note = Adeno-associated Virus
atgcagagggtgaacatgatcatggctgagagccctggcctgatcaccatctgcctgctgggctacctgctgtctgctgaatgtacagtttttcttgatcatgaaaatgccaacaaaattctgaatagaccaaagaggtataactctggcaagcttgaagagtttgtacaggggaatctggagagagagtgtatggaagagaagtgcagctttgaggaagccagagaagtgtttgaaaatacagagagaacaactgaattttggaagcagtatgtggatggtgatcaatgtgagagcaatccctgcttgaatggggggagctgtaaagatgatatcaacagctatgaatgttggtgtccctttggatttgaggggaaaaactgtgagcttgatgtgacctgtaatatcaagaatggcaggtgtgagcaattttgcaagaattctgctgataacaaagtggtctgtagctgcactgagggatataggctggctgaaaaccagaagagctgtgaacctgcagtgccttttccctgtgggagagtgtctgtgagccaaaccagcaagctgactagggctgaagcagtctttcctgatgtagattatgtgaatagcactgaggctgagacaatccttgacaatatcactcagagcacacagagcttcaatgacttcaccagggtggtaggaggggaggatgccaagcctgggcagttcccctggcaggtagtgctcaatggaaaagtggatgccttttgtggaggttcaattgtaaatgagaagtggattgtgactgcagcccactgtgtggaaactggagtcaagattactgtggtggctggagagcacaatattgaggaaactgagcacactgagcagaagaggaatgtgatcaggattatcccccaccacaactacaatgctgctatcaacaagtacaaccatgacattgccctcctggaactggatgaacccctggtcttgaacagctatgtgacacccatctgtattgctgataaagagtacaccaacatcttcttgaaatttgggtctggatatgtgtctggctggggcagggtgttccataaaggcaggtctgccctggtattgcagtatttgagggtgcctctggtggatagagcaacctgcttgctgagcaccaagtttacaatctacaacaatatgttctgtgcagggttccatgaaggtggtagagacagctgccagggagattctgggggtccccatgtgactgaggtggagggaaccagcttcctgactgggattatcagctggggtgaggagtgtgctatgaagggaaagtatgggatctacacaaaagtatccagatatgtgaactggattaaggagaaaaccaagctgacttga

SEQ ID NO: 11 - DNA, 1386 bp, unidentified
  source 1..1386: mol_type = other DNA; note = Adeno-associated Virus
atgcagcgcgtgaacatgatcatggccgagagccctggcctgattaccatctgcctgttaggatatctactcagtgctgaatgtacagtttttcttgatcatgaaaacgccaacaaaatcctgaaccggcccaagcggtacaactcaggcaagctggaagagttcgtgcagggcaacctggaacgggagtgcatggaagagaagtgcagcttcgaggaagcccgggaggtgttcgagaacaccgagcggaccaccgagttctggaagcagtacgtggacggcgaccagtgcgagtcaaacccctgcctgaacggcggcagctgcaaggacgatatcaacagctacgagtgctggtgccccttcggcttcgagggcaagaactgcgagctggacgtgacctgcaacatcaagaacggccgctgcgagcagttctgcaagaacagcgccgacaacaaggtggtgtgctcatgcactgagggctaccggctggccgagaaccagaagagctgcgagcccgccgtgcccttcccctgcggcagagtgtccgtgagccagaccagcaagctgaccagggccgaggccgtgttccctgacgtggactacgtgaactcaaccgaggccgagacaatcctggacaacatcacccagagcacccagtccttcaacgacttcacccgggtggtgggcggcgaggacgccaagcccggccagttcccttggcaggtggtgctgaacggcaaggtggacgccttctgcggcggctcaatcgtgaacgagaagtggatcgtgacagccgcccactgcgtggagacaggcgtgaagatcaccgtggtggccggcgaacacaatatcgaggaaaccgagcacaccgagcagaaacggaacgtgatccggattatcccccaccacaactacaacgccgccatcaacaagtacaaccacgatatcgccctgctggaactggacgagcctctggtgctgaattcatacgtgacccccatctgtatcgccgacaaagagtacaccaacatctttctgaagttcggcagcggctacgtgtccggctggggcagggtgttccacaagggccgcagcgccctggtgctgcagtacctgcgggtgcccctggtggacagagccacctgcctgcggtcaaccaagttcaccatctacaacaacatgttctgcgccggcttccacgagggcggcagggacagctgccagggcgacagcggcggaccccacgtgaccgaggtggagggcaccagctttctgaccggcatcatctcatggggcgaggaatgcgccatgaagggcaagtacggaatctacactaaggtgtcaagatacgtgaactggatcaaagagaaaaccaagctgacctga

SEQ ID NO: 12 - DNA, 11125 bp, unidentified
  source 1..11125: mol_type = other DNA; note = Adeno-associated Virus
cctgcaggcagctgcgcgctcgctcgctcactgaggccgcccgggcaaagcccgggcgtcgggcgacctttggtcgcccggcctcagtgagcgagcgagcgcgcagagagggagtggccaactccatcactaggggttcctgcggcctagtaggctcagaggcacacaggagtttctgggctcaccctgcccccttccaacccctcagttcccatcctccagcagctgtttgtgtgctgcctctgaagtccacactgaacaaacttcagcctactcatgtccctaaaatgggcaaacattgcaagcagcaaacagcaaacacacagccctccctgcctgctgaccttggagctggggcagaggtcagagacctctctgggcccatgccacctccaacatccactcgaccccttggaatttcggtggagaggagcagaggttgtcctggcgtggtttaggtagtgtgagaggggtacccggggatcttgctaccagtggaacagccactaaggattctgcagtgagagcagagggccagctaagtggtactctcccagagactgtctgactcacgccaccccctccaccttggacacaggacgctgtggtttctgagccaggtacaatgactcctttcggtaagtgcagtggaagctgtacactgcccaggcaaagcgtccgggcagcgtaggcgggcgactcagatcccagccagtggacttagcccctgtttgctcctccgataactggggtgaccttggttaatattcaccagcagcctcccccgttgcccctctggatccactgcttaaatacggacgaggacagggccctgtctcctcagcttcaggcaccaccactgacctgggacagtgaataccactttcacaatctgctagcaaaggttatgcagagggtgaacatgatcatggctgagagccctggcctgatcaccatctgcctgctgggctacctgctgtctgctgaatgtacaggtttgtttccttttttataatacattgagtatgcttgccttttagatatagaaatatctgattctgtcttcttcactaaattttgattacatgatttgacagcaatattgaagagtctaacagccagcacccaggttggtaagtactggttctttgttagctaggttttcttcttcttcacttttaaaactaaatagatggacaatgcttatgatgcaataaggtttaataaacactgttcagttcagtatttggtcatgtaattcctgttaaaaaacagtcatctccttggtttaaaaaaattaaaagtgggaaaacaaagaaatagcagaatatagtgaaaaaaaataaccacagtatttttgtttggacttaccactttgaaatcaaattgggaaacaaaagcacaaacagtggccttatttacacaaaaagtctgattttaagatatgtgacaattcaaggtttcagaagtatgtaaggaggtgtgtctctaattttttaaattatatatcttcaatttaaagttttagttaaaacataaagattaacctttcattagcaagctgttagttatcaccaaagcttttcatggattaggaaaaaatcattttgtctctatctcaaacatcttggagttgatatttggggaaacacaatactcagttgagttccctaggggagaaaagcaagcttaagaattgacacaaagagtaggaagttagctattgcaacatatatcactttgttttttcacaactacagtgactttatttatttcccagaggaaggcatacagggaagaaattatcccatttggacaaacagcatgttctcacagtaagcacttatcacacttacttgtcaactttctagaatcaaatctagtagctgacagtaccaggatcaggggtgccaaccctaagcacccccagaaagctgactggccctgtggttcccactccagacatgatgtcagctgtgaaatccacctccctggaccataattaggcttctgttcttcaggagacatttgttcaaagtcatttgggcaaccatattctgaaaacagcccagccagggtgatggatcactttgcaaagatcctcaatgagctattttcaagtgatgacaaagtgtgaagttaagggctcatttgagaactttctttttcatccaaagtaaattcaaatatgattagaaatctgaccttttattactggaattctcttgactaaaagtaaaattgaattttaattcctaaatctccatgtgtatacagtactgtgggaacatcacagattttggctccatgccctaaagagaaattggctttcagattatttggattaaaaacaaagactttcttaagagatgtaaaattttcatgatgttttcttttttgctaaaactaaagaattattcttttacatttcagtttttcttgatcatgaaaatgccaacaaaattctgaatagaccaaagaggtataactctggcaagcttgaagagtttgtacaggggaatctggagagagagtgtatggaagagaagtgcagctttgaggaagccagagaagtgtttgaaaatacagagagaacaactgaattttggaagcagtatgtggatggtgatcaatgtgagagcaatccctgcttgaatggggggagctgtaaagatgatatcaacagctatgaatgttggtgtccctttggatttgaggggaaaaactgtgagcttgatgtgacctgtaatatcaagaatggcaggtgtgagcaattttgcaagaattctgctgataacaaagtggtctgtagctgcactgagggatataggctggctgaaaaccagaagagctgtgaacctgcagtgccttttccctgtgggagagtgtctgtgagccaaaccagcaagctgactagggctgaagcagtctttcctgatgtagattatgtgaatagcactgaggctgagacaatccttgacaatatcactcagagcacacagagcttcaatgacttcaccagggtggtaggaggggaggatgccaagcctgggcagttcccctggcaggtagtgctcaatggaaaagtggatgccttttgtggaggttcaattgtaaatgagaagtggattgtgactgcagcccactgtgtggaaactggagtcaagattactgtggtggctggagagcacaatattgaggaaactgagcacactgagcagaagaggaatgtgatcaggattatcccccaccacaactacaatgctgctatcaacaagtacaaccatgacattgccctcctggaactggatgaacccctggtcttgaacagctatgtgacacccatctgtattgctgataaagagtacaccaacatcttcttgaaatttgggtctggatatgtgtctggctggggcagggtgttccataaaggcaggtctgccctggtattgcagtatttgagggtgcctctggtggatagagcaacctgcttgctgagcaccaagtttacaatctacaacaatatgttctgtgcagggttccatgaaggtggtagagacagctgccagggagattctgggggtccccatgtgactgaggtggagggaaccagcttcctgactgggattatcagctggggtgaggagtgtgctatgaagggaaagtatgggatctacacaaaagtatccagatatgtgaactggattaaggagaaaaccaagctgacttgatgaaagatggatttccaaggttaattcattggaattgaaaattaacagagatctagagctgaattcctgcagccagggggatcagcctctactgtgccttctagttgccagccatctgttgtttgcccctcccccttgccttccttgaccctggaaggtgccactcccactgtcctttcctaataaaatgaggaaattgcatcacattgtctgagtaggtgtcattctattctggggggtggggtggggcaggacagcaagggggaggattgggaagacaatagcaggcatgctggggatgcagtgggctctatggcttctgaggcagaaagaaccagctggggctcgagatccactagggccgcaggaacccctagtgatggagttggccactccctctctgcgcgctcgctcgctcactgaggccgcccgggctttgcccgggcggcctcagtgagcgagcgagcgcgcagctgcctgcaggggcagcttgaaggaaatactaaggcaaaggtactgcaagtgctcgcaacattcgcttatgcggattattgccgtagtgccgcgacgccgggggcaagatgcagagattgccatggtacaggccgtgcggttgatattgccaaaacagagctgtgggggagagttgtcgagaaagagtgcggaagatgcaaaggcgtcggctattcaaggatgccagcaagcgcagcatatcgcgctgtgacgatgctaatcccaaaccttacccaacccacctggtcacgcactgttaagccgctgtatgacgctctggtggtgcaatgccacaaagaagagtcaatcgcagacaacattttgaatgcggtcacacgttagcagcatgattgccacggatggcaacatattaacggcatgatattgacttattgaataaaattgggtaaatttgactcaacgatgggttaattcgctcgttgtggtagtgagatgaaaagaggcggcgcttactaccgattccgcctagttggtcacttcgacgtatcgtctggaactccaaccatcgcaggcagagaggtctgcaaaatgcaatcccgaaacagttcgcaggtaatagttagagcctgcataacggtttcgggattttttatatctgcacaacaggtaagagcattgagtcgataatcgtgaagagtcggcgagcctggttagccagtgctctttccgttgtgctgaattaagcgaataccggaagcagaaccggatcaccaaatgcgtacaggcgtcatcgccgcccagcaacagcacaacccaaactgagccgtagccactgtctgtcctgaattcattagtaatagttacgctgcggccttttacacatgaccttcgtgaaagcgggtggcaggaggtcgcgctaacaacctcctgccgttttgcccgtgcatatcggtcacgaacaaatctgattactaaacacagtagcctggatttgttctatcagtaatcgaccttattcctaattaaatagagcaaatccccttattgggggtaagacatgaagatgccagaaaaacatgacctgttggccgccattctcgcggcaaaggaacaaggcatcggggcaatccttgcgtttgcaatggcgtaccttcgcggcagatataatggcggtgcgtttacaaaaacagtaatcgacgcaacgatgtgcgccattatcgcctagttcattcgtgaccttctcgacttcgccggactaagtagcaatctcgcttatataacgagcgtgtttatcggctacatcggtactgactcgattggttcgcttatcaaacgcttcgctgctaaaaaagccggagtagaagatggtagaaatcaataatcaacgtaaggcgttcctcgatatgctggcgtggtcggagggaactgataacggacgtcagaaaaccagaaatcatggttatgacgtcattgtaggcggagagctatttactgattactccgatcaccctcgcaaacttgtcacgctaaacccaaaactcaaatcaacaggcgccggacgctaccagcttctttcccgttggtgggatgcctaccgcaagcagcttggcctgaaagacttctctccgaaaagtcaggacgctgtggcattgcagcagattaaggagcgtggcgctttacctatgattgatcgtggtgatatccgtcaggcaatcgaccgttgcagcaatatctgggcttcactgccgggcgctggttatggtcagttcgagcataaggctgacagcctgattgcaaaattcaaagaagcgggcggaacggtcagagagattgatgtatgagcagagtcaccgcgattatctccgctctggttatctgcatcatcgtctgcctgtcatgggctgttaatcattaccgtgataacgccattacctacaaagcccagcgcgacaaaaatgccagagaactgaagctggcgaacgcggcaattactgacatgcagatgcgtcagcgtgatgttgctgcgctcgatgcaaaatacacgaaggagttagctgatgctaaagctgaaaatgatgctctgcgtgatgatgttgccgctggtcgtcgtcggttgcacatcaaagcagtctgtcagtcagtgcgtgaagccaccaccgcctccggcgtggataatgcagcctccccccgactggcagacaccgctgaacgggattatttcaccctcagagagaggctgatcactatgcaaaaacaactggaaggaacccagaagtatattaatgagcagtgcagatagagttgcccatatcgatgggcaactcatgcaattattgtgagcaatacacacgcgcttccagcggagtataaatgcctaaagtaataaaaccgagcaatccatttacgaatgtttgctgggtttctgttttaacaacattttctgcgccgccacaaattttggctgcatcgacagttttcttctgcccaattccagaaacgaagaaatgatgggtgatggtttcctttggtgctactgctgccggtttgttttgaacagtaaacgtctgttgagcacatcctgtaataagcagggccagcgcagtagcgagtagcatttttttcatggtgttattcccgatgctttttgaagttcgcagaatcgtatgtgtagaaaattaaacaaaccctaaacaatgagttgaaatttcatattgttaatatttattaatgtatgtcaggtgcgatgaatcgtcattgtattcccggattaactatgtccacagccctgacggggaacttctctgcgggagtgtccgggaataattaaaacgatgcacacagggtttagcgcgtacacgtattgcattatgccaacgccccggtgctgacacggaagaaaccggacgttatgatttagcgtggaaagatttgtgtagtgttctgaatgctctcagtaaatagtaatgaattatcaaaggtatagtaatatcttttatgttcatggatatttgtaacccatcggaaaactcctgctttagcaagattttccctgtattgctgaaatgtgatttctcttgatttcaacctatcataggacgtttctataagatgcgtgtttcttgagaatttaacatttacaacctttttaagtccttttattaacacggtgttatcgttttctaacacgatgtgaatattatctgtggctagatagtaaatataatgtgagacgttgtgacgttttagttcagaataaaacaattcacagtctaaatcttttcgcacttgatcgaatatttctttaaaaatggcaacctgagccattggtaaaaccttccatgtgatacgagggcgcgtagtttgcattatcgtttttatcgtttcaatctggtctgacctccttgtgttttgttgatgatttatgtcaaatattaggaatgttttcacttaatagtattggttgcgtaacaaagtgcggtcctgctggcattctggagggaaatacaaccgacagatgtatgtaaggccaacgtgctcaaatcttcatacagaaagatttgaagtaatattttaaccgctagatgaagagcaagcgcatggagcgacaaaatgaataaagaacaatctgctgatgatccctccgtggatctgattcgtgtaaaaaatatgcttaatagcaccatttctatgagttaccctgatgttgtaattgcatgtatagaacataaggtgtctctggaagcattcagagcaattgaggcagcgttggtgaagcacgataataatatgaaggattattccctggtggttgactgatcaccataactgctaatcattcaaactatttagtctgtgacagagccaacacgcagtctgtcactgtcaggaaagtggtaaaactgcaactcaattactgcaatgccctcgtaattaagtgaatttacaatatcgtcctgttcggagggaagaacgcgggatgttcattcttcatcacttttaattgatgtatatgctctcttttctgacgttagtctccgacggcaggcttcaatgacccaggctgagaaattcccggaccctttttgctcaagagcgatgttaatttgttcaatcatttggttaggaaagcggatgttgcgggttgttgttctgcgggttctgttcttcgttgacatgaggttgccccgtattcagtgtcgctgatttgtattgtctgaagttgtttttacgttaagttgatgcagatcaattaatacgatacctgcgtcataattgattatttgacgtggtttgatggcctccacgcacgttgtgatatgtagatgataatcattatcactttacgggtcctttccggtgatccgacaggttacggggcggcgacctgcctgatgcggtattttctccttacgcatctgtgcggtatttcacaccgcatacgtcaaagcaaccatagtacgcgccctgtagcggcgcattaagcgcggcgggtgtggtggttacgcgcagcgtgaccgctacacttgccagcgccttagcgcccgctcctttcgctttcttcccttcctttctcgccacgttcgccggctttccccgtcaagctctaaatcgggggctccctttagggttccgatttagtgctttacggcacctcgaccccaaaaaacttgatttgggtgatggttcacgtagtgggccatcgccctgatagacggtttttcgccctttgacgttggagtccacgttctttaatagtggactcttgttccaaactggaacaacactcaactctatctcgggctattcttttgatttagacctgcaggcatgcaagcttggcactggccgtcgttttacaacgtcgtgactgggaaaaccctggcgttacccaacttaatcgccttgcagcacatccccctttcgccagctggcgtaatagcgaagaggcccgcaccgatcgcccttcccaacagttgcgcagcctgaatggcgaatgcgatttattcaacaaagccgccgtcccgtcaagtcagcgtaatgctctgccagtgttacaaccaattaaccaattctgattagaaaaactcatcgagcatcaaatgaaactgcaatttattcatatcaggattatcaataccatatttttgaaaaagccgtttctgtaatgaaggagaaaactcaccgaggcagttccataggatggcaagatcctggtatcggtctgcgattccgactcgtccaacatcaatacaacctattaatttcccctcgtcaaaaataaggttatcaagtgagaaatcaccatgagtgacgactgaatccggtgagaatggcaaaagcttatgcatttctttccagacttgttcaacaggccagccattacgctcgtcatcaaaatcactcgcatcaaccaaaccgttattcattcgtgattgcgcctgagcgagacgaaatacgcgatcgctgttaaaaggacaattacaaacaggaatcgaatgcaaccggcgcaggaacactgccagcgcatcaacaatattttcacctgaatcaggatattcttctaatacctggaatgctgttttcccggggatcgcagtggtgagtaaccatgcatcatcaggagtacggataaaatgcttgatggtcggaagaggcataaattccgtcagccagtttagtctgaccatctcatctgtaacatcattggcaacgctacctttgccatgtttcagaaacaactctggcgcatcgggcttcccatacaatcgatagattgtcgcacctgattgcccgacattatcgcgagcccatttatacccatataaatcagcatccatgttggaatttaatcgcggcttcgagcaagacgtttcccgttgaatatggctcataacaccccttgtattactgtttatgtaagcagacagttttattgttcatgatgatatatttttatcttgtgcaatgtaacatcagagattttgagacacaacgtggctttgttgaataaatcgaacttttgctgagttgaaggatcagatcacgcatcttcccgacaacgcagaccgttccgtggcaaagcaaaagttcaaaatcaccaactggtccacctacaacaaagctctcatcaaccgtggctccctcactttctggctggatgatggggcgattcaggcctggtatgagtcagcaacaccttcttcacgaggcagacctctcgacggagttccactgagcgtcagaccccgtagaaaagatcaaaggatcttcttgagatcctttttttctgcgcgtaatctgctgcttgcaaacaaaaaaaccaccgctaccagcggtggtttgtttgccggatcaagagctaccaactctttttccgaaggtaactggcttcagcagagcgcagataccaaatactgttcttctagtgtagccgtagttaggccaccacttcaagaactctgtagcaccgcctacatacctcgctctgctaatcctgttaccagtggctgctgccagtggcgataagtcgtgtcttaccgggttggactcaagacgatagttaccggataaggcgcagcggtcgggctgaacggggggttcgtgcacacagcccagcttggagcgaacgacctacaccgaactgagatacctacagcgtgagctatgagaaagcgccacgcttcccgaagggagaaaggcggacaggtatccggtaagcggcagggtcggaacaggagagcgcacgagggagcttccagggggaaacgcctggtatctttatagtcctgtcgggtttcgccacctctgacttgagcgtcgatttttgtgatgctcgtcaggggggcggagcctatggaaaaacgccagcaacgcggcctttttacggttcctggccttttgctggccttttgctcacatgt

SEQ ID NO: 13 - DNA, 141 bp, unidentified
  source 1..141: mol_type = other DNA; note = Adeno-associated Virus
cctgcaggcagctgcgcgctcgctcgctcactgaggccgcccgggcaaagcccgggcgtcgggcgacctttggtcgcccggcctcagtgagcgagcgagcgcgcagagagggagtggccaactccatcactaggggttcct

SEQ ID NO: 14 - DNA, 321 bp, unidentified
  source 1..321: mol_type = other DNA; note = Adeno-associated Virus
aggctcagaggcacacaggagtttctgggctcaccctgcccccttccaacccctcagttcccatcctccagcagctgtttgtgtgctgcctctgaagtccacactgaacaaacttcagcctactcatgtccctaaaatgggcaaacattgcaagcagcaaacagcaaacacacagccctccctgcctgctgaccttggagctggggcagaggtcagagacctctctgggcccatgccacctccaacatccactcgaccccttggaatttcggtggagaggagcagaggttgtcctggcgtggtttaggtagtgtgagaggg

SEQ ID NO: 15 - DNA, 397 bp, unidentified
  source 1..397: mol_type = other DNA; note = Adeno-associated Virus
gatcttgctaccagtggaacagccactaaggattctgcagtgagagcagagggccagctaagtggtactctcccagagactgtctgactcacgccaccccctccaccttggacacaggacgctgtggtttctgagccaggtacaatgactcctttcggtaagtgcagtggaagctgtacactgcccaggcaaagcgtccgggcagcgtaggcgggcgactcagatcccagccagtggacttagcccctgtttgctcctccgataactggggtgaccttggttaatattcaccagcagcctcccccgttgcccctctggatccactgcttaaatacggacgaggacagggccctgtctcctcagcttcaggcaccaccactgacctgggacagtgaat

SEQ ID NO: 16 - DNA, 29 bp, unidentified
  source 1..29: mol_type = other DNA; note = Adeno-associated Virus
accactttcacaatctgctagcaaaggtt

SEQ ID NO: 17 - DNA, 1438 bp, unidentified
  source 1..1438: mol_type = other DNA; note = Adeno-associated Virus
gtttgtttccttttttataatacattgagtatgcttgccttttagatatagaaatatctgattctgtcttcttcactaaattttgattacatgatttgacagcaatattgaagagtctaacagccagcacccaggttggtaagtactggttctttgttagctaggttttcttcttcttcacttttaaaactaaatagatggacaatgcttatgatgcaataaggtttaataaacactgttcagttcagtatttggtcatgtaattcctgttaaaaaacagtcatctccttggtttaaaaaaattaaaagtgggaaaacaaagaaatagcagaatatagtgaaaaaaaataaccacagtatttttgtttggacttaccactttgaaatcaaattgggaaacaaaagcacaaacagtggccttatttacacaaaaagtctgattttaagatatgtgacaattcaaggtttcagaagtatgtaaggaggtgtgtctctaattttttaaattatatatcttcaatttaaagttttagttaaaacataaagattaacctttcattagcaagctgttagttatcaccaaagcttttcatggattaggaaaaaatcattttgtctctatctcaaacatcttggagttgatatttggggaaacacaatactcagttgagttccctaggggagaaaagcaagcttaagaattgacacaaagagtaggaagttagctattgcaacatatatcactttgttttttcacaactacagtgactttatttatttcccagaggaaggcatacagggaagaaattatcccatttggacaaacagcatgttctcacagtaagcacttatcacacttacttgtcaactttctagaatcaaatctagtagctgacagtaccaggatcaggggtgccaaccctaagcacccccagaaagctgactggccctgtggttcccactccagacatgatgtcagctgtgaaatccacctccctggaccataattaggcttctgttcttcaggagacatttgttcaaagtcatttgggcaaccatattctgaaaacagcccagccagggtgatggatcactttgcaaagatcctcaatgagctattttcaagtgatgacaaagtgtgaagttaagggctcatttgagaactttctttttcatccaaagtaaattcaaatatgattagaaatctgaccttttattactggaattctcttgactaaaagtaaaattgaattttaattcctaaatctccatgtgtatacagtactgtgggaacatcacagattttggctccatgccctaaagagaaattggctttcagattatttggattaaaaacaaagactttcttaagagatgtaaaattttcatgatgttttcttttttgctaaaactaaagaattattcttttacatttcag

SEQ ID NO: 18 - DNA, 48 bp, unidentified
  source 1..48: mol_type = other DNA; note = Adeno-associated Virus
tgaaagatggatttccaaggttaattcattggaattgaaaattaacag

SEQ ID NO: 19 - DNA, 228 bp, unidentified
  source 1..228: mol_type = other DNA; note = Adeno-associated Virus
ctactgtgccttctagttgccagccatctgttgtttgcccctcccccttgccttccttgaccctggaaggtgccactcccactgtcctttcctaataaaatgaggaaattgcatcacattgtctgagtaggtgtcattctattctggggggtggggtggggcaggacagcaagggggaggattgggaagacaatagcaggcatgctggggatgcagtgggctctatgg

SEQ ID NO: 20 - DNA, 108 bp, unidentified
  source 1..108: mol_type = other DNA; note = Adeno-associated Virus
aggaacccctagtgatggagttggccactccctctctgcgcgctcgctcgctcactgaggccgcccgggctttgcccgggcggcctcagtgagcgagcgagcgcgcag

SEQ ID NO: 21 - DNA, 3631 bp, unidentified
  source 1..3631: mol_type = other DNA; note = Adeno-associated Virus
agcttgaaggaaatactaaggcaaaggtactgcaagtgctcgcaacattcgcttatgcggattattgccgtagtgccgcgacgccgggggcaagatgcagagattgccatggtacaggccgtgcggttgatattgccaaaacagagctgtgggggagagttgtcgagaaagagtgcggaagatgcaaaggcgtcggctattcaaggatgccagcaagcgcagcatatcgcgctgtgacgatgctaatcccaaaccttacccaacccacctggtcacgcactgttaagccgctgtatgacgctctggtggtgcaatgccacaaagaagagtcaatcgcagacaacattttgaatgcggtcacacgttagcagcatgattgccacggatggcaacatattaacggcatgatattgacttattgaataaaattgggtaaatttgactcaacgatgggttaattcgctcgttgtggtagtgagatgaaaagaggcggcgcttactaccgattccgcctagttggtcacttcgacgtatcgtctggaactccaaccatcgcaggcagagaggtctgcaaaatgcaatcccgaaacagttcgcaggtaatagttagagcctgcataacggtttcgggattttttatatctgcacaacaggtaagagcattgagtcgataatcgtgaagagtcggcgagcctggttagccagtgctctttccgttgtgctgaattaagcgaataccggaagcagaaccggatcaccaaatgcgtacaggcgtcatcgccgcccagcaacagcacaacccaaactgagccgtagccactgtctgtcctgaattcattagtaatagttacgctgcggccttttacacatgaccttcgtgaaagcgggtggcaggaggtcgcgctaacaacctcctgccgttttgcccgtgcatatcggtcacgaacaaatctgattactaaacacagtagcctggatttgttctatcagtaatcgaccttattcctaattaaatagagcaaatccccttattgggggtaagacatgaagatgccagaaaaacatgacctgttggccgccattctcgcggcaaaggaacaaggcatcggggcaatccttgcgtttgcaatggcgtaccttcgcggcagatataatggcggtgcgtttacaaaaacagtaatcgacgcaacgatgtgcgccattatcgcctagttcattcgtgaccttctcgacttcgccggactaagtagcaatctcgcttatataacgagcgtgtttatcggctacatcggtactgactcgattggttcgcttatcaaacgcttcgctgctaaaaaagccggagtagaagatggtagaaatcaataatcaacgtaaggcgttcctcgatatgctggcgtggtcggagggaactgataacggacgtcagaaaaccagaaatcatggttatgacgtcattgtaggcggagagctatttactgattactccgatcaccctcgcaaacttgtcacgctaaacccaaaactcaaatcaacaggcgccggacgctaccagcttctttcccgttggtgggatgcctaccgcaagcagcttggcctgaaagacttctctccgaaaagtcaggacgctgtggcattgcagcagattaaggagcgtggcgctttacctatgattgatcgtggtgatatccgtcaggcaatcgaccgttgcagcaatatctgggcttcactgccgggcgctggttatggtcagttcgagcataaggctgacagcctgattgcaaaattcaaagaagcgggcggaacggtcagagagattgatgtatgagcagagtcaccgcgattatctccgctctggttatctgcatcatcgtctgcctgtcatgggctgttaatcattaccgtgataacgccattacctacaaagcccagcgcgacaaaaatgccagagaactgaagctggcgaacgcggcaattactgacatgcagatgcgtcagcgtgatgttgctgcgctcgatgcaaaatacacgaaggagttagctgatgctaaagctgaaaatgatgctctgcgtgatgatgttgccgctggtcgtcgtcggttgcacatcaaagcagtctgtcagtcagtgcgtgaagccaccaccgcctccggcgtggataatgcagcctccccccgactggcagacaccgctgaacgggattatttcaccctcagagagaggctgatcactatgcaaaaacaactggaaggaacccagaagtatattaatgagcagtgcagatagagttgcccatatcgatgggcaactcatgcaattattgtgagcaatacacacgcgcttccagcggagtataaatgcctaaagtaataaaaccgagcaatccatttacgaatgtttgctgggtttctgttttaacaacattttctgcgccgccacaaattttggctgcatcgacagttttcttctgcccaattccagaaacgaagaaatgatgggtgatggtttcctttggtgctactgctgccggtttgttttgaacagtaaacgtctgttgagcacatcctgtaataagcagggccagcgcagtagcgagtagcatttttttcatggtgttattcccgatgctttttgaagttcgcagaatcgtatgtgtagaaaattaaacaaaccctaaacaatgagttgaaatttcatattgttaatatttattaatgtatgtcaggtgcgatgaatcgtcattgtattcccggattaactatgtccacagccctgacggggaacttctctgcgggagtgtccgggaataattaaaacgatgcacacagggtttagcgcgtacacgtattgcattatgccaacgccccggtgctgacacggaagaaaccggacgttatgatttagcgtggaaagatttgtgtagtgttctgaatgctctcagtaaatagtaatgaattatcaaaggtatagtaatatcttttatgttcatggatatttgtaacccatcggaaaactcctgctttagcaagattttccctgtattgctgaaatgtgatttctcttgatttcaacctatcataggacgtttctataagatgcgtgtttcttgagaatttaacatttacaacctttttaagtccttttattaacacggtgttatcgttttctaacacgatgtgaatattatctgtggctagatagtaaatataatgtgagacgttgtgacgttttagttcagaataaaacaattcacagtctaaatcttttcgcacttgatcgaatatttctttaaaaatggcaacctgagccattggtaaaaccttccatgtgatacgagggcgcgtagtttgcattatcgtttttatcgtttcaatctggtctgacctccttgtgttttgttgatgatttatgtcaaatattaggaatgttttcacttaatagtattggttgcgtaacaaagtgcggtcctgctggcattctggagggaaatacaaccgacagatgtatgtaaggccaacgtgctcaaatcttcatacagaaagatttgaagtaatattttaaccgctagatgaagagcaagcgcatggagcgacaaaatgaataaagaacaatctgctgatgatccctccgt

SEQ ID NO: 22 - DNA, 307 bp, unidentified
  source 1..307: mol_type = other DNA; note = Adeno-associated Virus
gcattaagcgcggcgggtgtggtggttacgcgcagcgtgaccgctacacttgccagcgccttagcgcccgctcctttcgctttcttcccttcctttctcgccacgttcgccggctttccccgtcaagctctaaatcgggggctccctttagggttccgatttagtgctttacggcacctcgaccccaaaaaacttgatttgggtgatggttcacgtagtgggccatcgccctgatagacggtttttcgccctttgacgttggagtccacgttctttaatagtggactcttgttccaaactggaacaa

SEQ ID NO: 23 - DNA, 813 bp, unidentified
  source 1..813: mol_type = other DNA; note = Adeno-associated Virus
gaaaaactcatcgagcatcaaatgaaactgcaatttattcatatcaggattatcaataccatatttttgaaaaagccgtttctgtaatgaaggagaaaactcaccgaggcagttccataggatggcaagatcctggtatcggtctgcgattccgactcgtccaacatcaatacaacctattaatttcccctcgtcaaaaataaggttatcaagtgagaaatcaccatgagtgacgactgaatccggtgagaatggcaaaagcttatgcatttctttccagacttgttcaacaggccagccattacgctcgtcatcaaaatcactcgcatcaaccaaaccgttattcattcgtgattgcgcctgagcgagacgaaatacgcgatcgctgttaaaaggacaattacaaacaggaatcgaatgcaaccggcgcaggaacactgccagcgcatcaacaatattttcacctgaatcaggatattcttctaatacctggaatgctgttttcccggggatcgcagtggtgagtaaccatgcatcatcaggagtacggataaaatgcttgatggtcggaagaggcataaattccgtcagccagtttagtctgaccatctcatctgtaacatcattggcaacgctacctttgccatgtttcagaaacaactctggcgcatcgggcttcccatacaatcgatagattgtcgcacctgattgcccgacattatcgcgagcccatttatacccatataaatcagcatccatgttggaatttaatcgcggcttcgagcaagacgtttcccgttgaatatggctcat

SEQ ID NO: 24 - DNA, 668 bp, unidentified
  source 1..668: mol_type = other DNA; note = Adeno-associated Virus
gtagaaaagatcaaaggatcttcttgagatcctttttttctgcgcgtaatctgctgcttgcaaacaaaaaaaccaccgctaccagcggtggtttgtttgccggatcaagagctaccaactctttttccgaaggtaactggcttcagcagagcgcagataccaaatactgttcttctagtgtagccgtagttaggccaccacttcaagaactctgtagcaccgcctacatacctcgctctgctaatcctgttaccagtggctgctgccagtggcgataagtcgtgtcttaccgggttggactcaagacgatagttaccggataaggcgcagcggtcgggctgaacggggggttcgtgcacacagcccagcttggagcgaacgacctacaccgaactgagatacctacagcgtgagctatgagaaagcgccacgcttcccgaagggagaaaggcggacaggtatccggtaagcggcagggtcggaacaggagagcgcacgagggagcttccagggggaaacgcctggtatctttatagtcctgtcgggtttcgccacctctgacttgagcgtcgatttttgtgatgctcgtcaggggggcggagcctatggaaaaacgccagcaacgcggcctttttacggttcctggccttttgctggccttttgctca

SEQ ID NO: 25 - DNA, 2824 bp, unidentified
  source 1..2824: mol_type = other DNA; note = Adeno-associated Virus
atgcagagggtgaacatgatcatggctgagagccctggcctgatcaccatctgcctgctgggctacctgctgtctgctgaatgtacaggtttgtttccttttttataatacattgagtatgcttgccttttagatatagaaatatctgattctgtcttcttcactaaattttgattacatgatttgacagcaatattgaagagtctaacagccagcacccaggttggtaagtactggttctttgttagctaggttttcttcttcttcacttttaaaactaaatagatggacaatgcttatgatgcaataaggtttaataaacactgttcagttcagtatttggtcatgtaattcctgttaaaaaacagtcatctccttggtttaaaaaaattaaaagtgggaaaacaaagaaatagcagaatatagtgaaaaaaaataaccacagtatttttgtttggacttaccactttgaaatcaaattgggaaacaaaagcacaaacagtggccttatttacacaaaaagtctgattttaagatatgtgacaattcaaggtttcagaagtatgtaaggaggtgtgtctctaattttttaaattatatatcttcaatttaaagttttagttaaaacataaagattaacctttcattagcaagctgttagttatcaccaaagcttttcatggattaggaaaaaatcattttgtctctatctcaaacatcttggagttgatatttggggaaacacaatactcagttgagttccctaggggagaaaagcaagcttaagaattgacacaaagagtaggaagttagctattgcaacatatatcactttgttttttcacaactacagtgactttatttatttcccagaggaaggcatacagggaagaaattatcccatttggacaaacagcatgttctcacagtaagcacttatcacacttacttgtcaactttctagaatcaaatctagtagctgacagtaccaggatcaggggtgccaaccctaagcacccccagaaagctgactggccctgtggttcccactccagacatgatgtcagctgtgaaatccacctccctggaccataattaggcttctgttcttcaggagacatttgttcaaagtcatttgggcaaccatattctgaaaacagcccagccagggtgatggatcactttgcaaagatcctcaatgagctattttcaagtgatgacaaagtgtgaagttaagggctcatttgagaactttctttttcatccaaagtaaattcaaatatgattagaaatctgaccttttattactggaattctcttgactaaaagtaaaattgaattttaattcctaaatctccatgtgtatacagtactgtgggaacatcacagattttggctccatgccctaaagagaaattggctttcagattatttggattaaaaacaaagactttcttaagagatgtaaaattttcatgatgttttcttttttgctaaaactaaagaattattcttttacatttcagtttttcttgatcatgaaaatgccaacaaaattctgaatagaccaaagaggtataactctggcaagcttgaagagtttgtacaggggaatctggagagagagtgtatggaagagaagtgcagctttgaggaagccagagaagtgtttgaaaatacagagagaacaactgaattttggaagcagtatgtggatggtgatcaatgtgagagcaatccctgcttgaatggggggagctgtaaagatgatatcaacagctatgaatgttggtgtccctttggatttgaggggaaaaactgtgagcttgatgtgacctgtaatatcaagaatggcaggtgtgagcaattttgcaagaattctgctgataacaaagtggtctgtagctgcactgagggatataggctggctgaaaaccagaagagctgtgaacctgcagtgccttttccctgtgggagagtgtctgtgagccaaaccagcaagctgactagggctgaagcagtctttcctgatgtagattatgtgaatagcactgaggctgagacaatccttgacaatatcactcagagcacacagagcttcaatgacttcaccagggtggtaggaggggaggatgccaagcctgggcagttcccctggcaggtagtgctcaatggaaaagtggatgccttttgtggaggttcaattgtaaatgagaagtggattgtgactgcagcccactgtgtggaaactggagtcaagattactgtggtggctggagagcacaatattgaggaaactgagcacactgagcagaagaggaatgtgatcaggattatcccccaccacaactacaatgctgctatcaacaagtacaaccatgacattgccctcctggaactggatgaacccctggtcttgaacagctatgtgacacccatctgtattgctgataaagagtacaccaacatcttcttgaaatttgggtctggatatgtgtctggctggggcagggtgttccataaaggcaggtctgccctggtattgcagtatttgagggtgcctctggtggatagagcaacctgcttgctgagcaccaagtttacaatctacaacaatatgttctgtgcagggttccatgaaggtggtagagacagctgccagggagattctgggggtccccatgtgactgaggtggagggaaccagcttcctgactgggattatcagctggggtgaggagtgtgctatgaagggaaagtatgggatctacacaaaagtatccagatatgtgaactggattaaggagaaaaccaagctgacttga

SEQ ID NO: 26 - DNA, 10659 bp, unidentified
  source 1..10659: mol_type = other DNA; note = Adeno-associated Virus
cctgcaggcagctgcgcgctcgctcgctcactgaggccgcccgggcaaagcccgggcgtcgggcgacctttggtcgcccggcctcagtgagcgagcgagcgcgcagagagggagtggccaactccatcactaggggttcctgcggcctagtaggctcagaggcacacaggagtttctgggctcaccctgcccccttccaacccctcagttcccatcctccagcagctgtttgtgtgctgcctctgaagtccacactgaacaaacttcagcctactcatgtccctaaaatgggcaaacattgcaagcagcaaacagcaaacacacagccctccctgcctgctgaccttggagctggggcagaggtcagagacctctctgggcccatgccacctccaacatccactcgaccccttggaatttcggtggagaggagcagaggttgtcctggcgtggtttaggtagtgtgagaggggtacccggggatcttgctaccagtggaacagccactaaggattctgcagtgagagcagagggccagctaagtggtactctcccagagactgtctgactcacgccaccccctccaccttggacacaggacgctgtggtttctgagccaggtacaatgactcctttcggtaagtgcagtggaagctgtacactgcccaggcaaagcgtccgggcagcgtaggcgggcgactcagatcccagccagtggacttagcccctgtttgctcctccgataactggggtgaccttggttaatattcaccagcagcctcccccgttgcccctctggatccactgcttaaatacggacgaggacagggccctgtctcctcagcttcaggcaccaccactgacctgggacagtgaataccactttcacaatctgctagcaaaggttatgcagagggtgaacatgatcatggctgagagccctggcctgatcaccatctgcctgctgggctacctgctgtctgctgaatgtacaggtttgtttccttttttataatacattgagtatgcttgccttttagatatagaaatatctgattctgtcttcttcactaaattttgattacatgatttgacagcaatattgaagagtctaacagccagcacccaggttggtaagtactggttctttgttagctaggttttcttcttcttcacttttaaaactaaatagatggacaatgcttatgatgcaataaggtttaataaacactgttcagttcagtatttggtcatgtaattcctgttaaaaaacagtcatctccttggtttaaaaaaattaaaagtgggaaaacaaagaaatagcagaatatagtgaaaaaaaataaccacagtatttttgtttggacttaccactttgaaatcaaattgggaaacaaaagcacaaacagtggccttatttacacaaaaagtctgattttaagatatgtgacaattcaaggtttcagaagtatgtaaggaggtgtgtctctaattttttaaattatatatcttcaatttaaagttttagttaaaacataaagattaacctttcattagcaacctcaatgagctattttcaagtgatgacaaagtgtgaagttaagggctcatttgagaactttctttttcatccaaagtaaattcaaatatgattagaaatctgaccttttattactggaattctcttgactaaaagtaaaattgaattttaattcctaaatctccatgtgtatacagtactgtgggaacatcacagattttggctccatgccctaaagagaaattggctttcagattatttggattaaaaacaaagactttcttaagagatgtaaaattttcatgatgttttcttttttgctaaaactaaagaattattcttttacatttcagtttttcttgatcatgaaaatgccaacaaaattctgaatagaccaaagaggtataactctggcaagcttgaagagtttgtacaggggaatctggagagagagtgtatggaagagaagtgcagctttgaggaagccagagaagtgtttgaaaatacagagagaacaactgaattttggaagcagtatgtggatggtgatcaatgtgagagcaatccctgcttgaatggggggagctgtaaagatgatatcaacagctatgaatgttggtgtccctttggatttgaggggaaaaactgtgagcttgatgtgacctgtaatatcaagaatggcaggtgtgagcaattttgcaagaattctgctgataacaaagtggtctgtagctgcactgagggatataggctggctgaaaaccagaagagctgtgaacctgcagtgccttttccctgtgggagagtgtctgtgagccaaaccagcaagctgactagggctgaagcagtctttcctgatgtagattatgtgaatagcactgaggctgagacaatccttgacaatatcactcagagcacacagagcttcaatgacttcaccagggtggtaggaggggaggatgccaagcctgggcagttcccctggcaggtagtgctcaatggaaaagtggatgccttttgtggaggttcaattgtaaatgagaagtggattgtgactgcagcccactgtgtggaaactggagtcaagattactgtggtggctggagagcacaatattgaggaaactgagcacactgagcagaagaggaatgtgatcaggattatcccccaccacaactacaatgctgctatcaacaagtacaaccatgacattgccctcctggaactggatgaacccctggtcttgaacagctatgtgacacccatctgtattgctgataaagagtacaccaacatcttcttgaaatttgggtctggatatgtgtctggctggggcagggtgttccataaaggcaggtctgccctggtattgcagtatttgagggtgcctctggtggatagagcaacctgcttgctgagcaccaagtttacaatctacaacaatatgttctgtgcagggttccatgaaggtggtagagacagctgccagggagattctgggggtccccatgtgactgaggtggagggaaccagcttcctgactgggattatcagctggggtgaggagtgtgctatgaagggaaagtatgggatctacacaaaagtatccagatatgtgaactggattaaggagaaaaccaagctgacttgatgaaagatggatttccaaggttaattcattggaattgaaaattaacagagatctagagctgaattcctgcagccagggggatcagcctctactgtgccttctagttgccagccatctgttgtttgcccctcccccttgccttccttgaccctggaaggtgccactcccactgtcctttcctaataaaatgaggaaattgcatcacattgtctgagtaggtgtcattctattctggggggtggggtggggcaggacagcaagggggaggattgggaagacaatagcaggcatgctggggatgcagtgggctctatggcttctgaggcagaaagaaccagctggggctcgagatccactagggccgcaggaacccctagtgatggagttggccactccctctctgcgcgctcgctcgctcactgaggccgggcgaccaaaggtcgcccgacgcccgggctttgcccgggcggcctcagtgagcgagcgagcgcgcagctgcctgcaggggcccatgggcagatgcaccacctgtctcagtgcaaagccctgcctaagtaggctggtcataagaccatgtgtctggctgtaactccaattgattgtcagcatcaataaaacttggccaacactgttatatactggtattgatagttacaactgaacatatttgtttaagcaattggaattaagaattcacatgcaatgatatcagggtccttctcctctggttagtgtattggggggaaattggacatctctcagctcagtaggctagttaggccaggatggatgacatccacagcccctgggcagagagattatgatgtagctagtctgactcctgacaaagacttgcttcctggagcttctactactttctggtggatggctaagaaatatggttgtgttcttttaagtctgaagagcattatttttgccaacccctgaccaaacatccttgccaaggaaaaggcctaaaatatatttgcatttaaagatattacaaactacttggttttggaatgtttggcctttcaggatcatagctatcaaaatattagctatttggggtatgagatgtctgcttggtcaaggacaagttcttaaagacatcatgttggggaataatggggaaaatgggaaggcttatgctctgagtaagacatctgagttatcatctgtcaaacatttttgttagtcatagtctaatgggagcctgttttccctctttaatatacattcacatctgaatttatgctcttcattgacaatgccagcccagaacaacagctcttaccctttggttttcttcctaacctttaactccaatgtaaccattacctgccatttcagtaaaaccattattctccctacttacccacccaagttgtacaataaagagtgtttgctctcactcatatacaaagcaaattcatttgtttgtgatgtacagcttgctatgcccacagatgtggtttgcctagtcctttgctctaggtcatttgactgggaacagatgggatgctcactttggtttttaatggttaactagtcattgaaatgcatttcatcaaataatcttagaggataattgtttaaatgtctgtccagactagctttgtagagccaggtgccattacacatgtcaccttcttatttctcttaattgaatttttatcatctgagataggaataatagagggctttttcaagtgaagatattactatagtctaaagaccttagtgtaacatcctggcccctaaggaaaaacaagttctggttcatacatataataactttgcatgttatctgccactgagatgtgtcctaatccaacagaaaggattgaatctctgtagctaggtgtacagggcaagagctgtacagggaacctttaaagatagcttcaggccaaagctgaggaaagtggatggagactggggaaaatgctaagacattttaaagattttctttaggtcaaaaatagaataagaaatagaccatttccctggacattttctgtaggttaatactgttaactattggtaaatgcatatgctacaacttaatatgtctgctttgtgagtttagcattgtctccttgtcattccagaaatgaaatggcaaatacatttaaatcagaactaaaaaggggaacagggtataaaggctcaatttagtcacatcatttccctttctcacccaccccctttaaaccagatgtttgccaatgcattaacaatgcagatgtttcctgaaagaaagtttagtaactcaagcagacaccttattttcttttcaagcagaaaagactatgagatggtggttgtggttgttctgggagggagaagatataaatgatacacattatttcaaatcatttcatgacctcactgcacacttatagttattgtacctgttgtctttttgctgtcaagcctagctaagatcatttggaatgttcaagatcactcatacatgcatgtgcacacatacacatgcacatatgttcactccctatttcatccacatgaactaagattactgatgtgtacagattcaaagcacttttattcttttccaaaggcaagaagctgagctactttccagaatagttgtgaaagaccctgtcatacttctgcattgtttcctccacaccacctccatccagttccttatgaatggttactggttttcaaaaatatgagataaattgagtgtataaaagtcatttttagacaaaatgaaacaggaaatgaaagaaaccagaatctctcctcatttgtggatgggccagctccaccatgtcatggttaatctgcagggaggaaatactagatttgattgcagatcagactgcagcaaacctgctgtgactaaggcatcaagagaaagcaagcaacagctggggcttcagtggtgaaaacattatatatctagctttgaaatatgaaatactgtttagcagtgtcacctagaaaagagtgtttcaaaatgctgatgcttcataagaacctttctcttcagagttgtttcttttatctttcaaattagccagggtgggaaataaagtgatcacttggtgaagaaatctcacaaagaagaacatagagagttcactttcatctggagtaatgaacagattgaacaaactagaaatggttagtctgttaaagaaaaggtgtaggtgagctgtttgcaagagccacaagggaaaggggaagacaacttctttgtggacttaagggtgaaagttgcaagcaggcaagaccattctgacctccattaagaaagccctttccaaccaacaaccactgggttggttactcaggttgggcagcattgggagcaaatgttgattgaacaaatgtttgtcagaattgttgacttaaagagctgttctgtcactggggacagcagcagctagatagccccattcagggagagggcatttgttcacctggccagagatcagagcaggctaagggactgctgggatcctgtccagctttgagaccctacagagccatgttcacctagcaggtatcccttctgaggtcactctcatttcttaccttattccagggctttcacctcagcttgccaggctggagccaagggccaaggcagcctcaccttgttggctatggtagcttcccaggagccccctatggttcaggaacagctctgcctgccccatcctgtttgctacctcctaaagccaaaggcactggtgggccaggccagcttctaaagtcacacaaggttagaaggttcctgacaggaagggcttgaggccaatggaaggaggtacttcagtttccctccagatgcccagtgatgggctcagagctccttgagaacttgggaaaggaagcagggtctctgaagaaatacttcaggagtagaaagaggaagctagagggttaaatgcactacacaggaacagaaatgagtttttcttagagttagtatatgtctagaggtgtagtaaactaaaacaagtcttgaattgcatacagccacttagggaagaaatgaaaacctttgaatattagtgaaaaaagggaaactgcaacccctgtattactagatagctttcatcaacagctcaaaacagacagatttttataggtttactgtgtgcactttaatacaagggcagtggttcagaactagtcaggtcctgaaaaggatttaccaaatgttgagtgtgccctctagtgttcacacttcccagctttcttcctataaaggtggatcaaggcacttgcttacaactggaactgaaatcctccaagtggaactagacattgagatggagaaaatattcattgtccactgtaattatgcaaggaatatccagttgagataatggacttgcctcttatctaataatacccaggctcaatgggtcactgctttgtccactttgcccaaaattcaagcacagctaagttgatattttaggacaaaggcagcttactatccagccagaggggagtagaatatggttaagagagagtggaaagaatgaatgagccctgctattcctcactgcctggatggctataagcacagcccttatggaggccttaggtcttgcttcataatattccagtttgaaaagggtttgaaaagacctcctagaaaaatcagtagtttttctcttttgagtaacatgtagcaaaaaaaatttcatcatgtaggtacagggaacaccctaataactattaatctcaaggagtcaagccagtgtgtttcctaatgtatctgctgtatccccatgaagcaaattttgccatcagagaaactgactcatggggaaaaaatccaaggacctcaaatcaccaaaagaagccattcctcagatttgcctaagcttaagcttccctgtctctcattgtgtgttgctttcaatgcagttacataaatggcttttttgtttatgcaccaaaaacactaattcatctgcaaagctataggtcaaagcaaccatagtatgcaccctgctagctggcgcattaagcgcggcgggtgtggtggttacgcgcagcgtgaccgctacacttgccagcgccttagcgcccgctcctttcgctttcttcccttcctttctcgccacgttcgccggctttccccgtcaagctctaaatcgggggctccctttagggttccgatttagtgctttacggcacctcgaccccaaaaaacttgatttgggtgatggttcacgtagtgggccatcgccctgatagacggtttttcgccctttgacgttggagtccacgttctttaatagtggactcttgttccaaactggaacaacactcaactctatctcgggctattcttttgatttagacctgcaggcatgcaagcttggcactggccgtcgttttacaacgtcgtgactgggaaaaccctggcgttacccaacttaatcgccttgcagcacatccccctttcgccagctggcgtaatagcgaagaggcccgcaccgatcgcccttcccaacagttgcgcagcctgaatggcgaatgcgatttattcaacaaagccgccgtcccgtcaagtcagcgtaatgctctgccagtgttacaaccaattaaccaattctgattagaaaaactcatcgagcatcaaatgaaactgcaatttattcatatcaggattatcaataccatatttttgaaaaagccgtttctgtaatgaaggagaaaactcaccgaggcagttccataggatggcaagatcctggtatcggtctgcgattccgactcgtccaacatcaatacaacctattaatttcccctcgtcaaaaataaggttatcaagtgagaaatcaccatgagtgacgactgaatccggtgagaatggcaaaagcttatgcatttctttccagacttgttcaacaggccagccattacgctcgtcatcaaaatcactcgcatcaaccaaaccgttattcattcgtgattgcgcctgagcgagacgaaatacgcgatcgctgttaaaaggacaattacaaacaggaatcgaatgcaaccggcgcaggaacactgccagcgcatcaacaatattttcacctgaatcaggatattcttctaatacctggaatgctgttttcccggggatcgcagtggtgagtaaccatgcatcatcaggagtacggataaaatgcttgatggtcggaagaggcataaattccgtcagccagtttagtctgaccatctcatctgtaacatcattggcaacgctacctttgccatgtttcagaaacaactctggcgcatcgggcttcccatacaatcgatagattgtcgcacctgattgcccgacattatcgcgagcccatttatacccatataaatcagcatccatgttggaatttaatcgcggcttcgagcaagacgtttcccgttgaatatggctcataacaccccttgtattactgtttatgtaagcagacagttttattgttcatgatgatatatttttatcttgtgcaatgtaacatcagagattttgagacacaacgtggctttgttgaataaatcgaacttttgctgagttgaaggatcagatcacgcatcttcccgacaacgcagaccgttccgtggcaaagcaaaagttcaaaatcaccaactggtccacctacaacaaagctctcatcaaccgtggctccctcactttctggctggatgatggggcgattcaggcctggtatgagtcagcaacaccttcttcacgaggcagacctctcgacggagttccactgagcgtcagaccccgtagaaaagatcaaaggatcttcttgagatcctttttttctgcgcgtaatctgctgcttgcaaacaaaaaaaccaccgctaccagcggtggtttgtttgccggatcaagagctaccaactctttttccgaaggtaactggcttcagcagagcgcagataccaaatactgttcttctagtgtagccgtagttaggccaccacttcaagaactctgtagcaccgcctacatacctcgctctgctaatcctgttaccagtggctgctgccagtggcgataagtcgtgtcttaccgggttggactcaagacgatagttaccggataaggcgcagcggtcgggctgaacggggggttcgtgcacacagcccagcttggagcgaacgacctacaccgaactgagatacctacagcgtgagctatgagaaagcgccacgcttcccgaagggagaaaggcggacaggtatccggtaagcggcagggtcggaacaggagagcgcacgagggagcttccagggggaaacgcctggtatctttatagtcctgtcgggtttcgccacctctgacttgagcgtcgatttttgtgatgctcgtcaggggggcggagcctatggaaaaacgccagcaacgcggcctttttacggttcctggccttttgctggccttttgctcacatgt

SEQ ID NO: 27 - protein, 601 aa, unidentified
  source 1..601: note = Adeno-associated Virus
TAPGKKRPVEPSPQRSPDSSTGIGKKGQQPAKKRLNFGQTGDSESVPDPQPIGEPPAAPSGVGPNTMAAGGGAPMADNNEGADGVGSSSGNWHCDSTWLGDRVITTSTRTWALPTYNNHLYKQISNGTSGGSTNDNTYFGYSTPWGYFDFNRFHCHFSPRDWQRLINNNWGFRPKRLNFKLFNIQVKEVTQNEGTKTIANNLTSTIQVFTDSEYQLPYVLGSAHQGCLPPFPADVFMIPQYGYLTLNNGSQAVGRSSFYCLEYFPSQMLRTGNNFEFSYNFEDVPFHSSYAHSQSLDRLMNPLIDQYLYYLSRTQSTGGTAGTQQLLFSQAGPNNMSAQAKNWLPGPCYRQQRVSTTLSQNNNSNFAWTGATKYHLNGRDSLVNPGVAMATHKDDEERFFPSSGVLMFGKQGAGKDNVDYSSVMLTSEEEIKTTNPVATEQYGVVADNLQQQNAAPIVGAVNSQGALPGMVWQNRDVYLQGPIWAKIPHTDGNFHPSPLMGGFGLKHPPPQILIKNTPVPADPPTTFNQAKLASFITQYSTGQVSVEIEWELQKENSKRWNPEIQYTSNYYKSTNVDFAVNTEGTYSEPRPIGTRYLTRNL